European Patent Specification EP 3 908 841 B1, published March 8, 2023. Title: IN VITRO METHOD FOR THE DIAGNOSIS OR PROGNOSIS OF NEURODEGENERATIVE DISORDERS. Applicant: Fundación Biomédica Galicia Sur (FBGS), SERVIZO GALEGO DE SAÚDE (SERGAS), Universidad de Vigo. The sequence listing filed with the application follows.

SEQUENCE LISTING (11 sequences)

SEQ ID NO: 1 - protein, 439 aa, Artificial sequence
  LRP1 48 KDa
MLTPPLLLLLPLLSALVAAAIDAPKTCSPKQFACRDQITCISKGWRCDGERDCPDGSDEAPEICPQSKAQRCQPNEHNCLGTELCVPMSRLCNGVQDCMDGSDEGPHCRELQGNCSRLGCQHHCVPTLDGPTCYCNSSFQLQADGKTCKDFDECSVYGTCSQLCTNTDGSFICGCVEGYLLQPDNRSCKAKNEPVDRPPVLLIANSQNILATYLSGAQVSTITPTSTRQTTAMDFSYANETVCWVHVGDSAAQTQLKCARMPGLKGFVDEHTINISLSLHHVEQMAIDWLTGNFYFVDDIDDRIFVCNRNGDTCVTLLDLELYNPKGIALDPAMGKVFFTDYGQIPKVERCDMDGQNRTKLVDSKIVFPHGITLDLVSRLVYWADAYLDYIEVVDYEGKGRQTIIQGILVRELLSEVLWGNHDPGPSGEGGSLCRGTVL

SEQ ID NO: 2 - protein, 183 aa, Artificial sequence
  LRP1 441, 179 KDa
NGQDNCGDGEDERDCPEVTCAPNQFQCSITKRCIPRVWVCDRDNDCVDGSDEPANCTQMTCGVDEFRCKDSGRCIPARWKCDGEDDCGDGSDEPKEECGEPRPHSRRKTVYLDERTCEPYQFRCKNNRCVPGRWQCDYDNDCGDNSDEESCTPRPCSESEFSCANGRCIAGRWKCDGDHDCAD

SEQ ID NO: 3 - protein, 4579 aa, Artificial sequence
  LRP1 498 KDa
LTVGADRDQQLCDPGEFLCHDHVTCVSQSWLCDGDPDCPDDSDESLDTCPEEVEIKCPLNHIACLGTNKCVHLSQLCNGVLDCPDGYDEGVHCQELLSNCQQLNCQYKCTMVRNSTRCYCEDGFEITEDGRSCKDQDECAVYGTCSQTCRNTHGSYTCSCVEGYLMQPDNRSCKAKIEPTDRPPILLIANFETIEVFYLNGSKMATLSSVNGNEIHTLDFIYNEDMICWIESRESSNQLKCIQITKAGGLTDEWTINILQSFHNVQQMAIDWLTRNLYFVDHVGDRIFVCNSNGSVCVTLIDLELHNPKAIAVDPIAGKLFFTDYGNVAKVERCDMDGMNRTRIIDSKTEQPAALALDLVNKLVYWVDLYLDYVGVVDYQGKNRHTVIQGRQVRHLYGITVFEDYLYATNSDNYNIVRINRFNGTDIHSLIKIENAWGIRIYQKRTQPTVRSHACEVDPYGMPGGCSHICLLSSSYKTRTCRCRTGFNLGSDGRSCKRPKNELFLFYGKGRPGIVRGMDLNTKIADEYMIPIENLVNPRALDFHAETNYIYFADTTSFLIGRQKIDGTERETILKDDLDNVEGIAVDWIGNNLYWTNDGHRKTINVARLEKASQSRKTLLEGEMSHPRGIVVDPVNGWMYWTDWEEDEIDDSVGRIEKAWMDGFNRQIFVTSKMLWPNGLTLDFHTNTLYWCDAYYDHIEKVFLNGTHRKIVYSGRELNHPFGLSHHGNYVFWTDYMNGSIFQLDLITSEVTLLRHERPPLFGLQIYDPRKQQGDNMCRVNNGGCSTLCLAIPGGRVCACADNQLLDENGTTCTFNPGEALPHICKAGEFRCKNRHCIQARWKCDGDDDCLDGSDEDSVNCFNHSCPDDQFKCQNNRCIPKRWLCDGANDCGSNEDESNQTCTARTCQVDQFSCGNGRCIPRAWLCDREDDCGDQTDEMASCEFPTCEPLTQFVCKSGRCISSKWHCDSDDDCGDGSDEVGCVHSCFDNQFRCSSGRCIPGHWACDGDNDCGDFSDEAQINCTKEEIHSPAGCNGNEFQCHPDGNCVPDLWRCDGEKDCEDGSDEKGCNGTIRLCDHKTKFSCWSTGRCINKAWVCDGDIDCEDQSDEDDCDSFLCGPPKHPCANDTSVCLQPEKLCNGKKDCPDGSDEGYLCDECSLNNGGCSNHCSVVPGRGIVCSCPEGLQLNKDNKTCEIVDYCSNHLKCSQVCEQHKHTVKCSCYEGWKLDVDGESCTSVDPFEAFIIFSIRHEIRRIDLHKRDYSLLVPGLRNTIALDFHFNQSLLYWTDVVEDRIYRGKLSESGGVSAIEVVVEHGLATPEGLTVDWIAGNIYWIDSNLDQIEVAKLDGSLRTTLIAGAMEHPRAIALDPRYGILFWTDWDANFPRIESASMSGAGRKTIYKDMKTGAWPNGLTVDHFEKRIVWTDARSDAIYSALYDGTNMIEIIRGHEYLSHPFAVSLYGSEVYWTDWRTNTLSKANKWTGQNVSVIQKTSAQPFDLQIYHPSRQPQAPNPCAANDGKGPCSHMCLINHNRSAACACPHLMKLSSDKKTCYEMKKFLLYARRSEIRGVDIDNPYFNFITAFTVPDIDDVTVIDFDASEERLYWTDIKTQTIKRAFINGTGLETVISRDIQSIRGLAVDWVSRNLYWISSEFDETQINVARLDGSLKTSIIHGIDKPQCLAAHPVRGKLYWTDGNTINMANMDGSNSKILFQNQKEPVGLSIDYVENKLYWISSGNGTINRCNLDGGNLEVIESMKEELTKATALTIMDKKLWWADQNLAQLGTCSKRDGRNPTILRNKTSGVVHMKVYDKEAQQGSNSCQLNNGGCSQLCLPTSETTRTCMCTVGYYLQKNRMSCQGIESFLMYSVHEGIRGIPLEPSDKMDALMPISGTSFAVGIDFHAENDTIYWTDMGFNKISRAKRDQTWKEDIITNGLGRVEGIAVDWIAGNIYWTDHGFNLIEVARLNGSFRYVIISQGLDQPRSIAVHPEKGLLFWTEWGQMPCIGKARLDGSEKVVLVSMGIAWPNGISIDYEENKLYWCDARTDKIERIDLETGGNREMVLSGSNVDMFSVAVFGAYIYWSDRAHANGSVRRGHKNDATETITMRTGLGVNLKEVKIFNRVREKGTNVCARDNGGCKQLCLYRGNSRRTCACAHGYLAEDGVTCLRHEGYLLYSGRTILKSIHLSDETNLNSPIRPYENPRYFKNVIALAFDYNQRRKGTNRIFYSDAHFGNIQLIKDNWEDRQVIVENVGSVEGLAYHRAWDTLYWTSSTTSSITRHTVDQTRPGAFDREAVITMSEDDHPHVLALDECQNLMFWTNWNEQHPSIMRSTLTGKNAQVVVSTDILTPNGLTIDYRAEKLYFSDGSLGKIERCEYDGSQRHVIVKSGPGTFLSLAVYDNYIFWSDWGRRAILRSNKYTGGDTKILRSDIPHQPMGIIAVANDTNSCELSPCALLNGGCHDLCLLTPNGRVNCSCRGDRILLEDNRCVTKNSSCNAYSEFECGNGECIDYQLTCDGIPHCKDKSDEKLLYCENRSCRRGFKPCYNRRCIPHGKLCDGENDCGDNSDELDCKVSTCATVEFRCADGTCIPRSARCNQNIDCADASDEKNCNNTDCTHFYKLGVKTTGFIRCNSTSLCVLPTWICDGSNDCGDYSDELKCPVQNKHKCEENYFSCPSGRCILNTWICDGQKDCEDGRDEFHCDSSCSWNQFACSAQKCISKHWICDGEDDCGDGLDESDSICGAITCAADMFSCQGSRACVPRHWLCDGERDCPDGSDELSTAGCAPNNTCDENAFMCHNKVCIPKQFVCDHDDDCGDGSDESPQCGYRQCGTEEFSCADGRCLLNTQWQCDGDFDCPDHSDEAPLNPKCKSAEQSCNSSFFMCKNGRCIPSGGLCDNKDDCGDGSDERNCHINECLSKKVSGCSQDCQDLPVSYKCKCWPGFQLKDDGKTCVDIDECSSGFPCSQQCINTYGTYKCLCTDGYEIQPDNPNGCKSLSDEEPFLILADHHEIRKISTDGSNYTLLKQGLNNVIAIDFDYREEFIYWIDSSRPNGSRINRMCLNGSDIKVVHNTAVPNALAVDWIGKNLYWSDTEKRIIEVSKLNGLYPTILVSKRLKFPRDLSLDPQAGYLYWIDCCEYPHIGRVGMDGTNQSVVIETKISRPMALTIDYVNRRLYWADENHIEFSNMDGSHRHKVPNQDIPGVIALTLFEDYIYWTDGKTKSLSRAHKTSGADRLSLIYSWHAITDIQVYHSYRQPDVSKHLCMINNGGCSHLCLLAPGKTHTCACPTNFYLAADNRTCLSNCTASQFRCKTDKCIPFWWKCDTVDDCGDGSDEPDDCPEFRCQPGRFQCGTGLCALPAFICDGENDCGDNSDELNCDTHVCLSGQFKCTKNQKCIPVNLRCNGQDDCGDEEDERDCPENSCSPDYFQCKTTKHCISKLWVCDEDPDCADASDEANCDKKTCGPHEFQCKNNNCIPDHWRCDSQNDCSDNSDEENCKPQTCTLKDFLCANGDCVSSRFWCDGDFDCADGSDERNCETSCSKDQFRCSNGQCIPAKWKCDGHEDCKYGEDEKSCEPASPTCSSREYICASDGCISASLKCNGEYDCADGSDEMDCVTECKEDQFRCKNKAHCIPIRWLCDGIHDCVDGSDEENCERGGNICRADEFLCNNSLCKLHFWVCDGEDDCGDNSDEAPDMCVKFLCPSTRPHRCRNNRICLQSEQMCNGIDECGDNSDEDHCGGKLTYKARPCKKDEFACSNKKCIPMDLQCDRLDDCGDGSDEQGCRIAPTEYTCEDNVNPCGDDAYCNQIKTSVFCRCKPGFQRNMKNRQCEDLNECLVFGTCSHQCINVEGSYKCVCDQNFQERNNTCIAEGSEDQVLYIANDTDILGFIYPFNYSGDHQQISHIEHNSRITGMDVYYQRDMIIWSTQFNPGGIFYKRIHGREKRQANSGLICPEFKRPRDIAVDWVAGNIYWTDHSRMHWFSYYTTHWTSLRYSINVGQLNGPNCTRLLTNMAGEPYAIAVNPKRGMMYWTVVGDHSHIEEAAMDGTLRRILVQKNLQRPTGLAVDYFSERIYWADFELSIIGSVLYDGSNSVVSVSSKQGLLHPHRIDIFEDYIYGAGPKNGVFRVQKFGHGSVEYLALNIDKTKGVLISHRYKQLDLPNPCLDLACEFLCLLNPSGATCVCPEGKYLINGTCNDDSLLDDSCKLTCENGGRCILNEKGDLRCHCWPSYSGERCEVNHCSNYCQNGGTCVPSVLGRPTCSCALGFTGPNCGKTVCEDFCQNGGTCIVTAGNQPYCHCQPEYTGDRCQYYVCHHYCVNSESCTIGDDGSVECVCPTRYEGPKCEVDKCVRCHGGHCIINKDSEDIFCNCTNGKIASSCQLCDGYCYNGGTCQLDPETNVPVCLCSTNWSGTQCERPAPKSSKSDHISTRSIAIIVPLVLLVTLITTLVIGLVLCKRKRRTKTIRRQPIINGGINVEIGNPSYNMYEVDHDHNDGGLLDPGFMIDPTKARYIGGGPSAFKLPHTAPPIYLNSDLKGPLTAGPTNYSNPVYAKLYMDGQNCRNSLGSVDERKELLPKKIEIGIRETVA

SEQ ID NO: 4 - protein, 3924 aa, Artificial sequence
  LRP1 515 KDa
AIDAPKTCSPKQFACRDQITCISKGWRCDGERDCPDGSDEAPEICPQSKAQRCQPNEHNCLGTELCVPMSRLCNGVQDCMDGSDEGPHCRELQGNCSRLGCQHHCVPTLDGPTCYCNSSFQLQADGKTCKDFDECSVYGTCSQLCTNTDGSFICGCVEGYLLQPDNRSCKAKNEPVDRPPVLLIANSQNILATYLSGAQVSTITPTSTRQTTAMDFSYANETVCWVHVGDSAAQTQLKCARMPGLKGFVDEHTINISLSLHHVEQMAIDWLTGNFYFVDDIDDRIFVCNRNGDTCVTLLDLELYNPKGIALDPAMGKVFFTDYGQIPKVERCDMDGQNRTKLVDSKIVFPHGITLDLVSRLVYWADAYLDYIEVVDYEGKGRQTIIQGILIEHLYGLTVFENYLYATNSDNANAQQKTSVIRVNRFNSTEYQVVTRVDKGGALHIYHQRRQPRVRSHACENDQYGKPGGCSDICLLANSHKARTCRCRSGFSLGSDGKSCKKPEHELFLVYGKGRPGIIRGMDMGAKVPDEHMIPIENLMNPRALDFHAETGFIYFADTTSYLIGRQKIDGTERETILKDGIHNVEGVAVDWMGDNLYWTDDGPKKTISVARLEKAAQTRKTLIEGKMTHPRAIVVDPLNGWMYWTDWEEDPKDSRRGRLERAWMDGSHRDIFVTSKTVLWPNGLSLDIPAGRLYWVDAFYDRIETILLNGTDRKIVYEGPELNHAFGLCHHGNYLFWTEYRSGSVYRLERGVGGAPPTVTLLRSERPPIFEIRMYDAQQQQVGTNKCRVNNGGCSSLCLATPGSRQCACAEDQVLDADGVTCLANPSYVPPPQCQPGEFACANSRCIQERWKCDGDNDCLDNSDEAPALCHQHTCPSDRFKCENNRCIPNRWLCDGDNDCGNSEDESNATCSARTCPPNQFSCASGRCIPISWTCDLDDDCGDRSDESASCAYPTCFPLTQFTCNNGRCININWRCDNDNDCGDNSDEAGCSHSCSSTQFKCNSGRCIPEHWTCDGDNDCGDYSDETHANCTNQATRPPGGCHTDEFQCRLDGLCIPLRWRCDGDTDCMDSSDEKSCEGVTHVCDPSVKFGCKDSARCISKAWVCDGDNDCEDNSDEENCESLACRPPSHPCANNTSVCLPPDKLCDGNDDCGDGSDEGELCDQCSLNNGGCSHNCSVAPGEGIVCSCPLGMELGPDNHTCQIQSYCAKHLKCSQKCDQNKFSVKCSCYEGWVLEPDGESCRSLDPFKPFIIFSNRHEIRRIDLHKGDYSVLVPGLRNTIALDFHLSQSALYWTDVVEDKIYRGKLLDNGALTSFEVVIQYGLATPEGLAVDWIAGNIYWVESNLDQIEVAKLDGTLRTTLLAGDIEHPRAIALDPRDGILFWTDWDASLPRIEAASMSGAGRRTVHRETGSGGWPNGLTVDYLEKRILWIDARSDAIYSARYDGSGHMEVLRGHEFLSHPFAVTLYGGEVYWTDWRTNTLAKANKWTGHNVTVVQRTNTQPFDLQVYHPSRQPMAPNPCEANGGQGPCSHLCLINYNRTVSCACPHLMKLHKDNTTCYEFKKFLLYARQMEIRGVDLDAPYYNYIISFTVPDIDNVTVLDYDAREQRVYWSDVRTQAIKRAFINGTGVETVVSADLPNAHGLAVDWVSRNLFWTSYDTNKKQINVARLDGSFKNAVVQGLEQPHGLVVHPLRGKLYWTDGDNISMANMDGSNRTLLFSGQKGPVGLAIDFPESKLYWISSGNHTINRCNLDGSGLEVIDAMRSQLGKATALAIMGDKLWWADQVSEKMGTCSKADGSGSVVLRNSTTLVMHMKVYDESIQLDHKGTNPCSVNNGDCSQLCLPTSETTRSCMCTAGYSLRSGQQACEGVGSFLLYSVHEGIRGIPLDPNDKSDALVPVSGTSLAVGIDFHAENDTIYWVDMGLSTISRAKRDQTWREDVVTNGIGRVEGIAVDWIAGNIYWTDQGFDVIEVARLNGSFRYVVISQGLDKPRAITVHPEKGYLFWTEWGQYPRIERSRLDGTERVVLVNVSISWPNGISVDYQDGKLYWCDARTDKIERIDLETGENREVVLSSNNMDMFSVSVFEDFIYWSDRTHANGSIKRGSKDNATDSVPLRTGIGVQLKDIKVFNRDRQKGTNVCAVANGGCQQLCLYRGRGQRACACAHGMLAEDGASCREYAGYLLYSERTILKSIHLSDERNLNAPVQPFEDPEHMKNVIALAFDYRAGTSPGTPNRIFFSDIHFGNIQQINDDGSRRITIVENVGSVEGLAYHRGWDTLYWTSYTTSTITRHTVDQTRPGAFERETVITMSGDDHPRAFVLDECQNLMFWTNWNEQHPSIMRAALSGANVLTLIEKDIRTPNGLAIDHRAEKLYFSDATLDKIERCEYDGSHRYVILKSEPVHPFGLAVYGEHIFWTDWVRRAVQRANKHVGSNMKLLRVDIPQQPMGIIAVANDTNSCELSPCRINNGGCQDLCLLTHQGHVNCSCRGGRILQDDLTCRAVNSSCRAQDEFECANGECINFSLTCDGVPHCKDKSDEKPSYCNSRRCKKTFRQCSNGRCVSNMLWCNGADDCGDGSDEIPCNKTACGVGEFRCRDGTCIGNSSRCNQFVDCEDASDEMNCSATDCSSYFRLGVKGVLFQPCERTSLCYAPSWVCDGANDCGDYSDERDCPGVKRPRCPLNYFACPSGRCIPMSWTCDKEDDCEHGEDETHCNKFCSEAQFECQNHRCISKQWLCDGSDDCGDGSDEAAHCEGKTCGPSSFSCPGTHVCVPERWLCDGDKDCADGADESIAAGCLYNSTCDDREFMCQNRQCIPKHFVCDHDRDCADGSDESPECEYPTCGPSEFRCANGRCLSSRQWECDGENDCHDQSDEAPKNPHCTSQEHKCNASSQFLCSSGRCVAEALLCNGQDDCGDSSDERGCHINECLSRKLSGCSQDCEDLKIGFKCRCRPGFRLKDDGRTCADVDECSTTFPCSQRCINTHGSYKCLCVEGYAPRGGDPHSCKAVTDEEPFLIFANRYYLRKLNLDGSNYTLLKQGLNNAVALDFDYREQMIYWTDVTTQGSMIRRMHLNGSNVQVLHRTGLSNPDGLAVDWVGGNLYWCDKGRDTIEVSKLNGAYRTVLVSSGLREPRALVVDVQNGYLYWTDWGDHSLIGRIGMDGSSRSVIVDTKITWPNGLTLDYVTERIYWADAREDYIEFASLDGSNRHVVLSQDIPHIFALTLFEDYVYWTDWETKSINRAHKTTGTNKTLLISTLHRPMDLHVFHALRQPDVPNHPCKVNNGGCSNLCLLSPGGGHKCACPTNFYLGSDGRTCVSNCTASQFVCKNDKCIPFWWKCDTEDDCGDHSDEPPDCPEFKCRPGQFQCSTGICTNPAFICDGDNDCQDNSDEANCDIHVCLPSQFKCTNTNRCIPGIFRCNGQDNCGDGEDERDCPEVTCAPNQFQCSITKRCIPRVWVCDRDNDCVDGSDEPANCTQMTCGVDEFRCKDSGRCIPARWKCDGEDDCGDGSDEPKEECDERTCEPYQFRCKNNRCVPGRWQCDYDNDCGDNSDEESCTPRPCSESEFSCANGRCIAGRWKCDGDHDCADGSDEKDCTPRCDMDQFQCKSGHCIPLRWRCDADADCMDGSDEEACGTGVRTCPLDEFQCNNTLCKPLAWKCDGEDDCGDNSDENPEECARFVCPPNRPFRCKNDRVCLWIGRQCDGTDNCGDGTDEEDCEPPTAHTTHCKDKKEFLCRNQRCLSSSLRCNMFDDCGDGSDEEDCSIDPKLTSCATNASICGDEARCVRTEKAAYCACRSGFHTVPGQPGCQDINECLRFGTCSQLCNNTKGGHLCSCARNFMKTHNTCKAEGSEYQVLYIADDNEIRSLFPGHPHSAYEQAFQGDESVRIDAMDVHVKAGRVYWTNWHTGTISYRSLPPAAPPTTSNRHRR

SEQ ID NO: 5 - protein, 4579 aa, Artificial sequence; identical to SEQ ID NO: 3
  LRP1 497,696 KDa

SEQ ID NO: 6 - protein, 2670 aa, Artificial sequence
  LRP1 293,591 KDa
VGSFLLYSVHEGIRGIPLDPNDKSDALVPVSGTSLAVGIDFHAENDTIYWVDMGLSTISRAKRDQTWREDVVTNGIGRVEGIAVDWIAGNIYWTDQGFDVIEVARLNGSFRYVVISQGLDKPRAITVHPEKGYLFWTEWGQYPRIERSRLDGTERVVLVNVSISWPNGISVDYQDGKLYWCDARTDKIERIDLETGENREVVLSSNNMDMFSVSVFEDFIYWSDRTHANGSIKRGSKDNATDSVPLRTGIGVQLKDIKVFNRDRQKGTNVCAVANGGCQQLCLYRGRGQRACACAHGMLAEDGASCREYAGYLLYSERTILKSIHLSDERNLNAPVQPFEDPEHMKNVIALAFDYRAGTSPGTPNRIFFSDIHFGNIQQINDDGSRRITIVENVGSVEGLAYHRGWDTLYWTSYTTSTITRHTVDQTRPGAFERETVITMSGDDHPRAFVLDECQNLMFWTNWNEQHPSIMRAALSGANVLTLIEKDIRTPNGLAIDHRAEKLYFSDATLDKIERCEYDGSHRYVILKSEPVHPFGLAVYGEHIFWTDWVRRAVQRANKHVGSNMKLLRVDIPQQPMGIIAVANDTNSCELSPCRINNGGCQDLCLLTHQGHVNCSCRGGRILQDDLTCRAVNSSCRAQDEFECANGECINFSLTCDGVPHCKDKSDEKPSYCNSRRCKKTFRQCSNGRCVSNMLWCNGADDCGDGSDEIPCNKTACGVGEFRCRDGTCIGNSSRCNQFVDCEDASDEMNCSATDCSSYFRLGVKGVLFQPCERTSLCYAPSWVCDGANDCGDYSDERDCPGVKRPRCPLNYFACPSGRCIPMSWTCDKEDDCEHGEDETHCNKFCSEAQFECQNHRCISKQWLCDGSDDCGDGSDEAAHCEGKTCGPSSFSCPGTHVCVPERWLCDGDKDCADGADESIAAGCLYNSTCDDREFMCQNRQCIPKHFVCDHDRDCADGSDESPECEYPTCGPSEFRCANGRCLSSRQWECDGENDCHDQSDEAPKNPHCTSPEHKCNASSQFLCSSGRCVAEELLCNGQDDCGDSSDERGCHINECLSHKLSGCSQDCEDLKIGFKCRCRPGFRLKDDGRTCADVDECSTTFPCSQRCINTHGSYKCLCVEGYAPRGGDPHSCKAVTDEEPFLIFANRYYLRKLNLDGSNYTLLKQGLNNAVALDFDYREQMIYWTDVTTQGSMIRRMHLNGSNVQVLHRTGLSNPDGLAVDWVGGNLYWCDKGRDTIEVSKLNGAYRTVLVSSGLREPRALVVDVQNGYLYWTDWGDHSLIGRIGMDGSSRSVIVDTKITWPNGLTLDYVTERIYWADAREDYIEFASLDGSNRHVVLSQDIPHIFALTLFEDYVYWTDWETKSINRAHKTTGTNKTLLISTLHRPMDLHVFHALRQPDVPNHPCKVNNGGCSNLCLLSPGGGHKCACPTNFYLGSDGRTCVSNCTASQFVCKNDKCIPFWWKCDTEDDCGDHSDEPPDCPEFKCRPGQFQCSTGICTNPAFICDGDNDCQDNSDEANCDIHVCLPSQFKCTNTNRCIPGIFRCNGQDNCGDGEDERDCPEVTCAPNQFQCSITKRCIPRVWVCDRDNDCVDGSDEPANCTQMTCGVDEFRCKDSGRCIPARWKCDGEDDCGDGSDEPKEECGEPRPHSRRKTVYLDERTCEPYQFRCKNNRCVPGRWQCDYDNDCGDNSDEESCTPRPCSESEFSCANGRCIAGRWKCDGDHDCADGSDEKDCTPRCDMDQFQCKSGHCIPLRWRCDADADCMDGSDEEACGTGVRTCPLDEFQCNNTLCKPLAWKCDGEDDCGDNSDENPEECARFVCPPNRPFRCKNDRVCLWIGRQCDGMDNCGDGTDEEDCEPPTAQTTHCKDKKEFLCRNQRCLSSSLRCNMFDDCGDGSDEEDCSIDPKLTSCATNASICGDEARCVRTEKAAYCACRSGFHTVPGQPGCQDINECLRFGTCSQLCNNTKGGHLCSCARNFMKTHNTCKAEGSEYQVLYIADDNEIRSLFPGHPHSAYEQAFQGDESVRIDAMDVHVKAGRVYWTNWHTGTISYRSLPPAAPPTTSNRHRRQIDRGVTHLNISGLKMPRGIAIDWVAGNVYWTDSGRDVIEVAQMKGENRKTLISGMIDEPHAIVVDPLRGTMYWSDWGNHPKIETAAMDGTLRETLVQDNIQWPTGLAVDYHNERLYWADAKLSVIGSIRLNGTDPIVAADSKRGLSHPFSIDVFEDYIYGVTYINNRVFKIHKFGHSPLVNLTGGLSHASDVVLYHQHKQPEVTNPCDRKKCEWLCLLSPSGPVCTCPNGKRLDNGTCVPVPSPTPPPDAPRPGTCNLQCFNGGSCFLNARRQPKCRCQPRYTGDKCELDQCWEHCRNGGTCAASPSGMPTCRCPTGFTGPKCTQQVCAGYCANNSTCTVNQGNQPQCRCLPGFLGDRCQYRQCSGYCENFGTCQMAADGSRQCRCTAYFEGPRCEVNKCSRCLEGACVVNKQSGDVTCNCTDGRVAPSCLTCVGHCSNGGSCTMNSKMMPECQCPPHMTGPRCEEHVFSQQQPGHIASILIPLLLLLLLLLVAGVVFWYKRRVQGAKGFQHQRMTNGAMNVEIGNPTYKMYEGGEPDDVGGLLDADFALDPDKPTNFTNPVYATLYMGGHGSRHSLASTDEKRELLGRGPEDEIGDPLA

SEQ ID NO: 7 - protein, 4544 aa, Artificial sequence
  pro-LRP1 504,276 KDa
MLTPPLLLLLPLLSALVAAAIDAPKTCSPKQFACRDQITCISKGWRCDGERDCPDGSDEAPEICPQSKAQRCQPNEHNCLGTELCVPMSRLCNGVQDCMDGSDEGPHCRELQGNCSRLGCQHHCVPTLDGPTCYCNSSFQLQADGKTCKDFDECSVYGTCSQLCTNTDGSFICGCVEGYLLQPDNRSCKAKNEPVDRPPVLLIANSQNILATYLSGAQVSTITPTSTRQTTAMDFSYANETVCWVHVGDSAAQTQLKCARMPGLKGFVDEHTINISLSLHHVEQMAIDWLTGNFYFVDDIDDRIFVCNRNGDTCVTLLDLELYNPKGIALDPAMGKVFFTDYGQIPKVERCDMDGQNRTKLVDSKIVFPHGITLDLVSRLVYWADAYLDYIEVVDYEGKGRQTIIQGILIEHLYGLTVFENYLYATNSDNANAQQKTSVIRVNRFNSTEYQVVTRVDKGGALHIYHQRRQPRVRSHACENDQYGKPGGCSDICLLANSHKARTCRCRSGFSLGSDGKSCKKPEHELFLVYGKGRPGIIRGMDMGAKVPDEHMIPIENLMNPRALDFHAETGFIYFADTTSYLIGRQKIDGTERETILKDGIHNVEGVAVDWMGDNLYWTDDGPKKTISVARLEKAAQTRKTLIEGKMTHPRAIVVDPLNGWMYWTDWEEDPKDSRRGRLERAWMDGSHRDIFVTSKTVLWPNGLSLDIPAGRLYWVDAFYDRIETILLNGTDRKIVYEGPELNHAFGLCHHGNYLFWTEYRSGSVYRLERGVGGAPPTVTLLRSERPPIFEIRMYDAQQQQVGTNKCRVNNGGCSSLCLATPGSRQCACAEDQVLDADGVTCLANPSYVPPPQCQPGEFACANSRCIQERWKCDGDNDCLDNSDEAPALCHQHTCPSDRFKCENNRCIPNRWLCDGDNDCGNSEDESNATCSARTCPPNQFSCASGRCIPISWTCDLDDDCGDRSDESASCAYPTCFPLTQFTCNNGRCININWRCDNDNDCGDNSDEAGCSHSCSSTQFKCNSGRCIPEHWTCDGDNDCGDYSDETHANCTNQATRPPGGCHTDEFQCRLDGLCIPLRWRCDGDTDCMDSSDEKSCEGVTHVCDPSVKFGCKDSARCISKAWVCDGDNDCEDNSDEENCESLACRPPSHPCANNTSVCLPPDKLCDGNDDCGDGSDEGELCDQCSLNNGGCSHNCSVAPGEGIVCSCPLGMELGPDNHTCQIQSYCAKHLKCSQKCDQNKFSVKCSCYEGWVLEPDGESCRSLDPFKPFIIFSNRHEIRRIDLHKGDYSVLVPGLRNTIALDFHLSQSALYWTDVVEDKIYRGKLLDNGALTSFEVVIQYGLATPEGLAVDWIAGNIYWVESNLDQIEVAKLDGTLRTTLLAGDIEHPRAIALDPRDGILFWTDWDASLPRIEAASMSGAGRRTVHRETGSGGWPNGLTVDYLEKRILWIDARSDAIYSARYDGSGHMEVLRGHEFLSHPFAVTLYGGEVYWTDWRTNTLAKANKWTGHNVTVVQRTNTQPFDLQVYHPSRQPMAPNPCEANGGQGPCSHLCLINYNRTVSCACPHLMKLHKDNTTCYEFKKFLLYARQMEIRGVDLDAPYYNYIISFTVPDIDNVTVLDYDAREQRVYWSDVRTQAIKRAFINGTGVETVVSADLPNAHGLAVDWVSRNLFWTSYDTNKKQINVARLDGSFKNAVVQGLEQPHGLVVHPLRGKLYWTDGDNISMANMDGSNRTLLFSGQKGPVGLAIDFPESKLYWISSGNHTINRCNLDGSGLEVIDAMRSQLGKATALAIMGDKLWWADQVSEKMGTCSKADGSGSVVLRNSTTLVMHMKVYDESIQLDHKGTNPCSVNNGDCSQLCLPTSETTRSCMCTAGYSLRSGQQACEGVGSFLLYSVHEGIRGIPLDPNDKSDALVPVSGTSLAVGIDFHAENDTIYWVDMGLSTISRAKRDQTWREDVVTNGIGRVEGIAVDWIAGNIYWTDQGFDVIEVARLNGSFRYVVISQGLDKPRAITVHPEKGYLFWTEWGQYPRIERSRLDGTERVVLVNVSISWPNGISVDYQDGKLYWCDARTDKIERIDLETGENREVVLSSNNMDMFSVSVFEDFIYWSDRTHANGSIKRGSKDNATDSVPLRTGIGVQLKDIKVFNRDRQKGTNVCAVANGGCQQLCLYRGRGQRACACAHGMLAEDGASCREYAGYLLYSERTILKSIHLSDERNLNAPVQPFEDPEHMKNVIALAFDYRAGTSPGTPNRIFFSDIHFGNIQQINDDGSRRITIVENVGSVEGLAYHRGWDTLYWTSYTTSTITRHTVDQTRPGAFERETVITMSGDDHPRAFVLDECQNLMFWTNWNEQHPSIMRAALSGANVLTLIEKDIRTPNGLAIDHRAEKLYFSDATLDKIERCEYDGSHRYVILKSEPVHPFGLAVYGEHIFWTDWVRRAVQRANKHVGSNMKLLRVDIPQQPMGIIAVANDTNSCELSPCRINNGGCQDLCLLTHQGHVNCSCRGGRILQDDLTCRAVNSSCRAQDEFECANGECINFSLTCDGVPHCKDKSDEKPSYCNSRRCKKTFRQCSNGRCVSNMLWCNGADDCGDGSDEIPCNKTACGVGEFRCRDGTCIGNSSRCNQFVDCEDASDEMNCSATDCSSYFRLGVKGVLFQPCERTSLCYAPSWVCDGANDCGDYSDERDCPGVKRPRCPLNYFACPSGRCIPMSWTCDKEDDCEHGEDETHCNKFCSEAQFECQNHRCISKQWLCDGSDDCGDGSDEAAHCEGKTCGPSSFSCPGTHVCVPERWLCDGDKDCADGADESIAAGCLYNSTCDDREFMCQNRQCIPKHFVCDHDRDCADGSDESPECEYPTCGPSEFRCANGRCLSSRQWECDGENDCHDQSDEAPKNPHCTSQEHKCNASSQFLCSSGRCVAEALLCNGQDDCGDSSDERGCHINECLSRKLSGCSQDCEDLKIGFKCRCRPGFRLKDDGRTCADVDECSTTFPCSQRCINTHGSYKCLCVEGYAPRGGDPHSCKAVTDEEPFLIFANRYYLRKLNLDGSNYTLLKQGLNNAVALDFDYREQMIYWTDVTTQGSMIRRMHLNGSNVQVLHRTGLSNPDGLAVDWVGGNLYWCDKGRDTIEVSKLNGAYRTVLVSSGLREPRALVVDVQNGYLYWTDWGDHSLIGRIGMDGSSRSVIVDTKITWPNGLTLDYVTERIYWADAREDYIEFASLDGSNRHVVLSQDIPHIFALTLFEDYVYWTDWETKSINRAHKTTGTNKTLLISTLHRPMDLHVFHALRQPDVPNHPCKVNNGGCSNLCLLSPGGGHKCACPTNFYLGSDGRTCVSNCTASQFVCKNDKCIPFWWKCDTEDDCGDHSDEPPDCPEFKCRPGQFQCSTGICTNPAFICDGDNDCQDNSDEANCDIHVCLPSQFKCTNTNRCIPGIFRCNGQDNCGDGEDERDCPEVTCAPNQFQCSITKRCIPRVWVCDRDNDCVDGSDEPANCTQMTCGVDEFRCKDSGRCIPARWKCDGEDDCGDGSDEPKEECDERTCEPYQFRCKNNRCVPGRWQCDYDNDCGDNSDEESCTPRPCSESEFSCANGRCIAGRWKCDGDHDCADGSDEKDCTPRCDMDQFQCKSGHCIPLRWRCDADADCMDGSDEEACGTGVRTCPLDEFQCNNTLCKPLAWKCDGEDDCGDNSDENPEECARFVCPPNRPFRCKNDRVCLWIGRQCDGTDNCGDGTDEEDCEPPTAHTTHCKDKKEFLCRNQRCLSSSLRCNMFDDCGDGSDEEDCSIDPKLTSCATNASICGDEARCVRTEKAAYCACRSGFHTVPGQPGCQDINECLRFGTCSQLCNNTKGGHLCSCARNFMKTHNTCKAEGSEYQVLYIADDNEIRSLFPGHPHSAYEQAFQGDESVRIDAMDVHVKAGRVYWTNWHTGTISYRSLPPAAPPTTSNRHRRQIDRGVTHLNISGLKMPRGIAIDWVAGNVYWTDSGRDVIEVAQMKGENRKTLISGMIDEPHAIVVDPLRGTMYWSDWGNHPKIETAAMDGTLRETLVQDNIQWPTGLAVDYHNERLYWADAKLSVIGSIRLNGTDPIVAADSKRGLSHPFSIDVFEDYIYGVTYINNRVFKIHKFGHSPLVNLTGGLSHASDVVLYHQHKQPEVTNPCDRKKCEWLCLLSPSGPVCTCPNGKRLDNGTCVPVPSPTPPPDAPRPGTCNLQCFNGGSCFLNARRQPKCRCQPRYTGDKCELDQCWEHCRNGGTCAASPSGMPTCRCPTGFTGPKCTQQVCAGYCANNSTCTVNQGNQPQCRCLPGFLGDRCQYRQCSGYCENFGTCQMAADGSRQCRCTAYFEGSRCEVNKCSRCLEGACVVNKQSGDVTCNCTDGRVAPSCLTCVGHCSNGGSCTMNSKMMPECQCPPHMTGPRCEEHVFSQQQPGHIASILIPLLLLLLLVLVAGVVFWYKRRVQGAKGFQHQRMTNGAMNVEIGNPTYKMYEGGEPDDVGGLLDADFALDPDKPTNFTNPVYATLYMGGHGSRHSLASTDEKRELLGRGPEDEIGDPLA

SEQ ID NO: 8 - protein, 1225 aa, Artificial sequence
  LRP2 220 KDa
MDRGPAAVACTLLLALVACLAPASGQECDSAHFRCGSGHCIPADWRCDGTKDCSDDADEIGCAVVTCQQGYFKCQSEGQCIPNSWVCDQDQDCDDGSDERQDCSQSTCSSHQITCSNGQCIPSEYRCDHVRDCPDGADENDCQYPTCEQLTCDNGACYNTSQKCDWKVDCRDSSDEINCTEICLHNEFSCGNGECIPRAYVCDHDNDCQDGSDEHACNYPTCGGYQFTCPSGRCIYQNWVCDGEDDCKDNGDEDGCESGPHDVHKCSPREWSCPESGRCISIYKVCDGILDCPGREDENNTSTGKYCSMTLCSALNCQYQCHETPYGGACFCPPGYIINHNDSRTCVEFDDCQIWGICDQKCESRPGRHLCHCEEGYILERGQYCKANDSFGEASIIFSNGRDLLIGDIHGRSFRILVESQNRGVAVGVAFHYHLQRVFWTDTVQNKVFSVDINGLNIQEVLNVSVETPENLAVDWVNNKIYLVETKVNRIDMVNLDGSYRVTLITENLGHPRGIAVDPTVGKTVVHGGSLIPHPFGVSLFEGQVFFTDWTKMAVLKANKFTETNPQVYYQASLRPYGVTVYHSLRQPYATNPCKDNNGGCEQVCVLSHRTDNDGLGFRCKCTFGFQLDTDERHCIGREILAANRVENVESLAFDWISKNLYWTDSHYKSISVMRLADKTRRTVVQYLNNPRSVVVHPFAGYLFFTDWFRPAKIMRAWSDGSHLLPVINTTLGWPNGLAIDWAASRLYWVDAYFDKIEHSTFDGLDRRRLGHIEQMTHPFGLAIFGEHLFFTDWRLGAIIRVRKADGGEMTVIRSGIAYILHLKSYDVNIQTGSNACNQPTHPNGDCSHFCFPVPNFQRVCGCPYGMRLASNHLTCEGDPTNEPPTEQCGLFSFPCKNGRCVPNYYLCDGVDDCHDNSDEQLCGTLNNTCSSSAFTCGHGECIPAHWRCDKRNDCVDGSDEHNCPTHAPASCLDTQYTCDNHQCISKNWVCDTDNDCGDGSDEKNCNSTETCQPSQFNCPNHRCIDLSFVCDGDKDCVDGSDEVGCVLNCTASQFKCASGDKCIGVTNRCDGVFDCSDNSDEAGCPTRPPGMCHSDEFQCQEDGICIPNFWECDGHPDCLYGSDEHNACVPKTCPSSYFHCDNGNCIHRAWLCDRDNDCGDMSDEKDCPTQPFRCPSWQWQCLGHNICVNLSVVCDGIFDCPNGTDESPLCSKFPDHSLLAINSF

SEQ ID NO: 9 - protein, 4544 aa, Artificial sequence; identical to SEQ ID NO: 7
  LRP1

SEQ ID NO: 10 - protein, 347 aa, Artificial sequence
  LRP2BP
MKLTSEKLPKNPFYASVSQYAAKNQKFFQWKKEKTDYTHANLVDKALQLLKERILKGDTLAYFLRGQLYFEEGWYEEALEQFEEIKEKDHQATYQLGVMYYDGLGTTLDAEKGVDYMKKILDSPCPKARHLKFAAAYNLGRAYYEGKGVKRSNEEAERLWLIAADNGNPKASVKAQSMLGLYYSTKEPKELEKAFYWHSEACGNGNLESQGALGLMYLYGQGIRQDTEAALQCLREAAERGNVYAQGNLVEYYYKMKFFTKCVAFSKRIADYDEVHDIPMIAQVTDCLPEFIGRGMAMASFYHARCLQLGLGITRDETTAKHYYSKACRLNPALADELHSLLIRQRI

SEQ ID NO: 11 - protein, 601 aa, Artificial sequence
  LRP1 85 KDa
QIDRGVTHLNISGLKMPRGIAIDWVAGNVYWTDSGRDVIEVAQMKGENRKTLISGMIDEPHAIVVDPLRGTMYWSDWGNHPKIETAAMDGTLRETLVQDNIQWPTGLAVDYHNERLYWADAKLSVIGSIRLNGTDPIVAADSKRGLSHPFSIDVFEDYIYGVTYINNRVFKIHKFGHSPLVNLTGGLSHASDVVLYHQHKQPEVTNPCDRKKCEWLCLLSPSGPVCTCPNGKRLDNGTCVPVPSPTPPPDAPRPGTCNLQCFNGGSCFLNARRQPKCRCQPRYTGDKCELDQCWEHCRNGGTCAASPSGMPTCRCPTGFTGPKCTQQVCAGYCANNSTCTVNQGNQPQCRCLPGFLGDRCQYRQCSGYCENFGTCQMAADGSRQCRCTAYFEGSRCEVNKCSRCLEGACVVNKQSGDVTCNCTDGRVAPSCLTCVGHCSNGGSCTMNSKMMPECQCPPHMTGPRCEEHVFSQQQPGHIASILIPLLLLLLLVLVAGVVFWYKRRVQGAKGFQHQRMTNGAMNVEIGNPTYKMYEGGEPDDVGGLLDADFALDPDKPTNFTNPVYATLYMGGHGSRHSLASTDEKRELLGRGPEDEIGDPLA